European Patent Specification EP 3 896 083 B1, published March 1, 2023. Title: FC FUSION PROTEINS COMPRISING NOVEL LINKERS OR ARRANGEMENTS. Applicant: BRISTOL-MYERS SQUIBB COMPANY. Application EP. The sequence listing filed with the application follows.

SEQUENCE LISTING (154 sequences)

SEQ ID NO: 1 - protein, 94 aa, Homo sapiens
VSDVPRDLEVVAATPTSLLISWDAPAVTVRYYRITYGETGGNSPVQEFTVPGSKSTATISGLKPGVDYTITVYAVTGRGDSPASSKPISINYRT

SEQ ID NO: 2 - protein, 137 aa, Artificial Sequence
  source: /note="Description of Artificial Sequence: Synthetic polypeptide"
  MOD_RES (7)..(21): Any amino acid
  misc_feature (7)..(21): /note="This region may encompass 1 to 15 residues"
  MOD_RES (26)..(45): Any amino acid
  misc_feature (26)..(45): /note="This region may encompass 2 to 20 residues"
  MOD_RES (54)..(73): Any amino acid
  misc_feature (54)..(73): /note="This region may encompass 2 to 20 residues"
  MOD_RES (79)..(88): Any amino acid
  misc_feature (79)..(88): /note="This region may encompass 2 to 20 residues"
  MOD_RES (92)..(101): Any amino acid
  misc_feature (92)..(101): /note="This region may encompass 2 to 20 residues"
  MOD_RES (111)..(130): Any amino acid
  misc_feature (111)..(130): /note="This region may encompass 2 to 20 residues"
  source: /note="see specification as filed for detailed description of substitutions and preferred embodiments"
EVVAATXXXXXXXXXXXXXXXSLLIXXXXXXXXXXXXXXXXXXXXYYRITYGEXXXXXXXXXXXXXXXXXXXXQEFTVXXXXXXXXXXATIXXXXXXXXXXDYTITVYAVXXXXXXXXXXXXXXXXXXXXISINYRT

SEQ ID NO: 3 - protein, 98 aa, Artificial Sequence
  source: /note="Description of Artificial Sequence: Synthetic polypeptide"
  MOD_RES (13)..(22): Any amino acid
  misc_feature (13)..(22): /note="This region may encompass 2 to 20 residues"
  MOD_RES (43)..(52): Any amino acid
  misc_feature (43)..(52): /note="This region may encompass 2 to 20 residues"
  MOD_RES (72)..(91): Any amino acid
  misc_feature (72)..(91): /note="This region may encompass 2 to 20 residues"
  source: /note="see specification as filed for detailed description of substitutions and preferred embodiments"
EVVAATPTSLLIXXXXXXXXXXYYRITYGETGGNSPVQEFTVXXXXXXXXXXATISGLKPGVDYTITVYAVXXXXXXXXXXXXXXXXXXXXISINYRT

SEQ ID NO: 4 - protein, 10 aa, Artificial Sequence
  source: /note="Description of Artificial Sequence: Synthetic peptide"
MGVSDVPRDL

SEQ ID NO: 5 - protein, 8 aa, Artificial Sequence
  source: /note="Description of Artificial Sequence: Synthetic peptide"
VSDVPRDL

SEQ ID NO: 6 - protein, 9 aa, Artificial Sequence
  source: /note="Description of Artificial Sequence: Synthetic peptide"
GVSDVPRDL

SEQ ID NO: 7 - protein, 9 aa, Artificial Sequence
  source: /note="Description of Artificial Sequence: Synthetic peptide"
  VARIANT (1)..(1): /replace=" "
  VARIANT (2)..(2): /replace=" "
  misc_feature (1)..(2): /note="Residues given in the sequence have no preference with respect to those in the annotations for said positions"
MGSDVPRDL

SEQ ID NO: 8 - protein, 8 aa, Artificial Sequence
  source: /note="Description of Artificial Sequence: Synthetic peptide"
  VARIANT (1)..(1): /replace=" "
  VARIANT (2)..(2): /replace=" "
  misc_feature (1)..(2): /note="Residues given in the sequence have no preference with respect to those in the annotations for said positions"
MGDVPRDL

SEQ ID NO: 9 - protein, 7 aa, Artificial Sequence
  source: /note="Description of Artificial Sequence: Synthetic peptide"
  VARIANT (1)..(1): /replace=" "
  VARIANT (2)..(2): /replace=" "
  misc_feature (1)..(2): /note="Residues given in the sequence have no preference with respect to those in the annotations for said positions"
MGVPRDL

SEQ ID NO: 10 - protein, 6 aa, Artificial Sequence
  source: /note="Description of Artificial Sequence: Synthetic peptide"
  VARIANT (1)..(1): /replace=" "
  VARIANT (2)..(2): /replace=" "
  misc_feature (1)..(2): /note="Residues given in the sequence have no preference with respect to those in the annotations for said positions"
MGPRDL

SEQ ID NO: 11 - protein, 5 aa, Artificial Sequence
  source: /note="Description of Artificial Sequence: Synthetic peptide"
  VARIANT (1)..(1): /replace=" "
  VARIANT (2)..(2): /replace=" "
  misc_feature (1)..(2): /note="Residues given in the sequence have no preference with respect to those in the annotations for said positions"
MGRDL

SEQ ID NO: 12 - protein, 4 aa, Artificial Sequence
  source: /note="Description of Artificial Sequence: Synthetic peptide"
  VARIANT (1)..(1): /replace=" "
  VARIANT (2)..(2): /replace=" "
  misc_feature (1)..(2): /note="Residues given in the sequence have no preference with respect to those in the annotations for said positions"
MGDL

SEQ ID NO: 13 - protein, 4 aa, Artificial Sequence
  source: /note="Description of Artificial Sequence: Synthetic peptide"
EIEK

SEQ ID NO: 14 - protein, 5 aa, Artificial Sequence
  source: /note="Description of Artificial Sequence: Synthetic peptide"
EGSGC

SEQ ID NO: 15 - protein, 7 aa, Artificial Sequence
  source: /note="Description of Artificial Sequence: Synthetic peptide"
EIEKPCQ

SEQ ID NO: 16 - protein, 7 aa, Artificial Sequence
  source: /note="Description of Artificial Sequence: Synthetic peptide"
EIEKPSQ

SEQ ID NO: 17 - protein, 5 aa, Artificial Sequence
  source: /note="Description of Artificial Sequence: Synthetic peptide"
EIEKP

SEQ ID NO: 18 - protein, 6 aa, Artificial Sequence
  source: /note="Description of Artificial Sequence: Synthetic peptide"
EIEKPS

SEQ ID NO: 19 - protein, 6 aa, Artificial Sequence
  source: /note="Description of Artificial Sequence: Synthetic peptide"
EIEKPC

SEQ ID NO: 20 - protein, 7 aa, Artificial Sequence
  source: /note="Description of Artificial Sequence: Synthetic peptide"
EIDKPSQ

SEQ ID NO: 21 - protein, 9 aa, Artificial Sequence
  source: /note="Description of Artificial Sequence: Synthetic peptide"
EIDKPSQLE

SEQ ID NO: 22 - protein, 330 aa, Homo sapiens [sequence omitted]

SEQ ID NO: 23 - protein, 16 aa, Homo sapiens
DKTHTCPPCPAPELLG

SEQ ID NO: 24 - protein, 24 aa, Artificial Sequence
  source: /note="Description of Artificial Sequence: Synthetic peptide"
EPKSSDKTHTCPPCPAPELLGGPS

SEQ ID NO: 25 - protein, 24 aa, Artificial Sequence
  source: /note="Description of Artificial Sequence: Synthetic peptide"
EPKSSDKTHTCPPCPAPELLGGSS

SEQ ID NO: 26 - protein, 24 aa, Artificial Sequence
  source: /note="Description of Artificial Sequence: Synthetic peptide"
EPKSSGSTHTCPPCPAPELLGGSS

SEQ ID NO: 27 - protein, 19 aa, Artificial Sequence
  source: /note="Description of Artificial Sequence: Synthetic peptide"
DKTHTCPPCPAPELLGGPS

SEQ ID NO: 28 - protein, 19 aa, Artificial Sequence
  source: /note="Description of Artificial Sequence: Synthetic peptide"
DKTHTCPPCPAPELLGGSS

SEQ ID NO: 29 - protein, 20 aa, Artificial Sequence
  source: /note="Description of Artificial Sequence: Synthetic peptide"
METDTLLLWVLLLWVPGSTG

SEQ ID NO: 30 - protein, 330 aa, Artificial Sequence
  source: /note="Description of Artificial Sequence: Synthetic polypeptide"
GVSDVPRDLEVVAATPTSLLISWVPPSDDYGYYRITYGETGGNSPVQEFTVPIGKGTATISGLKPGVDYTITVYAVEFPWPHAGYYHRPISINYRTEIEPKSSGSTHTCPPCPAPELLGGSSVFLFPPKPKDTLMISRTPEVTCVVVDVSHEDPEVKFNWYVDGVEVHNAKTKPREEQYNSTYRVVSVLTVLHQDWLNGKEYKCKVSNKALPAPIEKTISKAKGQPREPQVYTLPPSRDELTKNQVSLTCLVKGFYPSDIAVEWESNGQPENNYKTTPPVLDSDGSFFLYSKLTVDKSRWQQGNVFSCSVMHEALHNHYTQKSLSLSPGK

SEQ ID NO: 31 - protein, 208 aa, Homo sapiens
VFLFPPKPKDTLMISRTPEVTCVVVDVSHEDPEVKFNWYVDGVEVHNAKTKPREEQYNSTYRVVSVLTVLHQDWLNGKEYKCKVSNKALPAPIEKTISKAKGQPREPQVYTLPPSRDELTKNQVSLTCLVKGFYPSDIAVEWESNGQPENNYKTTPPVLDSDGSFFLYSKLTVDKSRWQQGNVFSCSVMHEALHNHYTQKSLSLSPGK

SEQ ID NO: 32 - protein, 10 aa, Artificial Sequence
  source: /note="Description of Artificial Sequence: Synthetic peptide"
GSGSGSGSGS

SEQ ID NO: 33 - protein, 12 aa, Artificial Sequence
  source: /note="Description of Artificial Sequence: Synthetic peptide"
GSGSGSGSGSGS

SEQ ID NO: 34 - protein, 20 aa, Artificial Sequence
  source: /note="Description of Artificial Sequence: Synthetic peptide"
GSGSGSGSGSGSGSGSGSGS

SEQ ID NO: 35 - protein, 15 aa, Artificial Sequence
  source: /note="Description of Artificial Sequence: Synthetic peptide"
GGGGSGGGGSGGGGS

SEQ ID NO: 36 - protein, 15 aa, Artificial Sequence
  source: /note="Description of Artificial Sequence: Synthetic peptide"
GGGGSGGGGSGGGSG

SEQ ID NO: 37 - protein, 7 aa, Artificial Sequence
  source: /note="Description of Artificial Sequence: Synthetic peptide"
AGGGGSG

SEQ ID NO: 38 - protein, 8 aa, Artificial Sequence
  source: /note="Description of Artificial Sequence: Synthetic peptide"
AGGGGSGG

SEQ ID NO: 39 - protein, 3 aa, Artificial Sequence
  source: /note="Description of Artificial Sequence: Synthetic peptide"
GPG

SEQ ID NO: 40 - protein, 7 aa, Artificial Sequence
  source: /note="Description of Artificial Sequence: Synthetic peptide"
GPGPGPG

SEQ ID NO: 41 - protein, 11 aa, Artificial Sequence
  source: /note="Description of Artificial Sequence: Synthetic peptide"
GPGPGPGPGPG

SEQ ID NO: 42 - protein, 6 aa, Artificial Sequence
  source: /note="Description of Artificial Sequence: Synthetic peptide"
PAPAPA

SEQ ID NO: 43 - protein, 12 aa, Artificial Sequence
  source: /note="Description of Artificial Sequence: Synthetic peptide"
PAPAPAPAPAPA

SEQ ID NO: 44 - protein, 18 aa, Artificial Sequence
  source: /note="Description of Artificial Sequence: Synthetic peptide"
PAPAPAPAPAPAPAPAPA

SEQ ID NO: 45 - protein, 8 aa, Artificial Sequence
  source: /note="Description of Artificial Sequence: Synthetic peptide"
QPDEPGGS

SEQ ID NO: 46 - protein, 17 aa, Artificial Sequence
  source: /note="Description of Artificial Sequence: Synthetic peptide"
ELQLEESAAEAQDGELD

SEQ ID NO: 47 - protein, 6 aa, Artificial Sequence
  source: /note="Description of Artificial Sequence: Synthetic peptide"
TVAAPS

SEQ ID NO: 48 - protein, 9 aa, Artificial Sequence
  source: /note="Description of Artificial Sequence: Synthetic peptide"
QPDEPGGSG

SEQ ID NO: 49 - protein, 18 aa, Artificial Sequence
  source: /note="Description of Artificial Sequence: Synthetic peptide"
ELQLEESAAEAQDGELDG

SEQ ID NO: 50 - protein, 7 aa, Artificial Sequence
  source: /note="Description of Artificial Sequence: Synthetic peptide"
TVAAPSG

SEQ ID NO: 51 - protein, 31 aa, Artificial Sequence
  source: /note="Description of Artificial Sequence: Synthetic polypeptide"
SCSVADWQMPPPYVVLDLPQETLEEETPGAN

SEQ ID NO: 52 - protein, 31 aa, Artificial Sequence
  source: /note="Description of Artificial Sequence: Synthetic polypeptide"
SCCVADWQMPPPYVVLDLPQETLEEETPGAN

SEQ ID NO: 53 - protein, 26 aa, Artificial Sequence
  source: /note="Description of Artificial Sequence: Synthetic peptide"
DWQMPPPYVVLDLPQETLEEETPGAN

SEQ ID NO: 54 - protein, 31 aa, Artificial Sequence; identical to SEQ ID NO: 52
  source: /note="Description of Artificial Sequence: Synthetic polypeptide"

SEQ ID NO: 55 - protein, 27 aa, Artificial Sequence
  source: /note="Description of Artificial Sequence: Synthetic peptide"
YLAMTPLIPQSKDENSDDYTTFDDVGS

SEQ ID NO: 56 - protein, 15 aa, Artificial Sequence
  source: /note="Description of Artificial Sequence: Synthetic peptide"
ELDVCVEEAEGEAPW

SEQ ID NO: 57 - protein, 18 aa, Artificial Sequence
  source: /note="Description of Artificial Sequence: Synthetic peptide"
ELQLEESCAEAQDGELDG

SEQ ID NO: 58 - protein, 13 aa, Artificial Sequence
  source: /note="Description of Artificial Sequence: Synthetic peptide"
EGEVSADEEGFEN

SEQ ID NO: 59 - protein, 19 aa, Artificial Sequence
  source: /note="Description of Artificial Sequence: Synthetic peptide"
KPTHVNVSVVMAEVDGTCY

SEQ ID NO: 60 - protein, 19 aa, Artificial Sequence
  source: /note="Description of Artificial Sequence: Synthetic peptide"
KPTHVNVSVVMAEVDGTCY

SEQ ID NO: 61 - protein, 9 aa, Artificial Sequence
  source: /note="Description of Artificial Sequence: Synthetic peptide"
YVTDHGPMK

SEQ ID NO: 62 - protein, 18 aa, Artificial Sequence
  source: /note="Description of Artificial Sequence: Synthetic peptide"
PTLYNVSLVMSDTAGTCY

SEQ ID NO: 63 - protein, 31 aa, Artificial Sequence
  source: /note="Description of Artificial Sequence: Synthetic polypeptide"
  VARIANT (2)..(2): /replace="Ala" or "Gly"
  misc_feature (2)..(2): /note="Residue given in the sequence has no preference with respect to those in the annotation for said position"
SSSVADWQMPPPYVVLDLPQETLEEETPGAN

SEQ ID NO: 64 - protein, 31 aa, Artificial Sequence; identical to SEQ ID NO: 63
  source: /note="Description of Artificial Sequence: Synthetic polypeptide"
  VARIANT (2)..(3): /replace="Ala" or "Gly"
  misc_feature (2)..(3): /note="Residues given in the sequence have no preference with respect to those in the annotations for said positions"

SEQ ID NO: 65 - protein, 31 aa, Artificial Sequence; identical to SEQ ID NO: 63
  source: /note="Description of Artificial Sequence: Synthetic polypeptide"
  VARIANT (2)..(3): /replace="Ala" or "Gly"
  misc_feature (2)..(3): /note="Residues given in the sequence have no preference with respect to those in the annotations for said positions"

SEQ ID NO: 66 - protein, 15 aa, Artificial Sequence [sequence omitted]

SEQ ID NO: 67 - protein, 18 aa, Artificial Sequence
  source: /note="Description of Artificial Sequence: Synthetic peptide"
  VARIANT (8)..(8): /replace="Ala" or "Gly"
  misc_feature (8)..(8): /note="Residue given in the sequence has no preference with respect to those in the annotation for said position"
ELQLEESSAEAQDGELDG

SEQ ID NO: 68 - protein, 19 aa, Artificial Sequence
  source: /note="Description of Artificial Sequence: Synthetic peptide"
  VARIANT (18)..(18): /replace="Ala" or "Gly"
  misc_feature (18)..(18): /note="Residue given in the sequence has no preference with respect to those in the annotation for said position"
KPTHVNVSVVMAEVDGTSY

SEQ ID NO: 69 - protein, 19 aa, Artificial Sequence
  source: /note="Description of Artificial Sequence: Synthetic peptide"
  VARIANT (18)..(18): /replace="Ala" or "Gly"
  misc_feature (18)..(18): /note="Residue given in the sequence has no preference with respect to those in the annotation for said position"
KPTHVNVSVVMAEVDGTSY

SEQ ID NO: 70 - protein, 18 aa, Artificial Sequence
  source: /note="Description of Artificial Sequence: Synthetic peptide"
  VARIANT (17)..(17): /replace="Ala" or "Gly"
  misc_feature (17)..(17): /note="Residue given in the sequence has no preference with respect to those in the annotation for said position"
PTLYNVSLVMSDTAGTSY

SEQ ID NO: 71 - protein, 7 aa, Artificial Sequence
  source: /note="Description of Artificial Sequence: Synthetic peptide"
PSTSTST

SEQ ID NO: 72 - protein, 104 aa, Artificial Sequence
  source: /note="Description of Artificial Sequence: Synthetic polypeptide"
MGVSDVPRDLEVVAATPTSLLISWVPPSDDYGYYRITYGETGGNSPVQEFTVPIGKGTATISGLKPGVDYTITVYAVEFPWPHAGYYHRPISINYRTEIEKPCQ

SEQ ID NO: 73 - DNA, 314 bp, Artificial Sequence
  source: /note="Description of Artificial Sequence: Synthetic polynucleotide"
atgggagtttctgatgtgccgcgcgacctggaagtggttgctgccacccccaccagcctgctgatcagctgggtcccgccttcagatgattacggttattaccgcatcacttacggcgaaacaggaggcaatagccctgtccaggagttcactgtgcctattggtaaaggaacagctaccatcagcggccttaaacctggcgttgattataccatcactgtgtatgctgtcgagtttccgtggccacatgctggttactatcatcggccaatttccattaattaccgcacagaaattgagaaaccatgccagtg

SEQ ID NO: 74 - protein, 104 aa, Artificial Sequence
  source: /note="Description of Artificial Sequence: Synthetic polypeptide"
MGVSDVPRDLEVVAATPTSLLISWVPPSDDYGYYRITYGETGGNSPVQEFTVPIGKGTATISGLKPGVDYTITVYAVEFPWPHAGYYHRPISINYRTEIDKPSQ

SEQ ID NO: 75 - DNA, 330 bp, Artificial Sequence
  source: /note="Description of Artificial Sequence: Synthetic polynucleotide"
atgggagtttctgatgtgccgcgcgacctggaagtggttgctgccacccccaccagcctgctgatcagctgggtcccgccttcagatgattacggttattaccgcatcacttacggcgaaacaggaggcaatagccctgtccaggagttcactgtgcctattggtaaaggaacagctaccatcagcggccttaaacctggcgttgattataccatcactgtgtatgctgtcgagtttccgtggccacatgctggttactatcatcggccaatttccattaattaccgcacagaaattgacaaaccatcccagcaccatcaccaccaccac

SEQ ID NO: 76 - protein, 101 aa, Artificial Sequence
  source: /note="Description of Artificial Sequence: Synthetic polypeptide"
MGVSDVPRDLEVVAATPTSLLISWVPPSDDYGYYRITYGETGGNSPVQEFTVPIGKGTATISGLKPGVDYTITVYAVEFPWPHAGYYHRPISINYRTGSGC

SEQ ID NO: 77 - DNA, 321 bp, Artificial Sequence
  source: /note="Description of Artificial Sequence: Synthetic polynucleotide"
atgggagtttctgatgtgccgcgcgacctggaagtggttgctgccacccccaccagcctgctgatcagctgggtcccgccttcagatgattacggttattaccgcatcacttacggcgaaacaggaggcaatagccctgtccaggagttcactgtgcctattggtaaaggaacagctaccatcagcggccttaaacctggcgttgattataccatcactgtgtatgctgtcgagtttccgtggccacatgctggttactatcatcggccaatttccattaattaccgcacaggtagcggttgccaccatcaccaccatcac

SEQ ID NO: 78 - protein, 104 aa, Artificial Sequence
  source: /note="Description of Artificial Sequence: Synthetic polypeptide"
MGVSDVPRDLEVVAATPTSLLISWPPPSHGYGYYRITYGETGGNSPVQEFTVPPGKGTATISGLKPGVDYTITVYAVEYPYKHSGYYHRPISINYRTEIDKPCQ

SEQ ID NO: 79 - DNA, 330 bp, Artificial Sequence
  source: /note="Description of Artificial Sequence: Synthetic polynucleotide"
atgggagtttctgatgtgccgcgcgacctggaagtggttgctgccacccccaccagcctgctgatcagctggccgccgccgtctcatggttacggttattaccgcatcacttacggcgaaacaggaggcaatagccctgtccaggagttcactgtgccgcctggtaaaggtacagctaccatcagcggccttaaacctggcgttgattataccatcactgtgtatgctgtcgaatacccgtacaaacattctggttactaccatcgtccaatttccattaattaccgcacagaaattgacaaaccatgccagcaccatcaccaccaccac

SEQ ID NO: 80 - protein, 25 aa, Artificial Sequence
  source: /note="Description of Artificial Sequence: Synthetic peptide"
GGGGSGGGGSGGGGSGGGGSGGGGS

SEQ ID NO: 81 - protein, 5 aa, Artificial Sequence
  source: /note="Description of Artificial Sequence: Synthetic peptide"
QPDEP

SEQ ID NO: 82 - protein, 7 aa, Artificial Sequence
  source: /note="Description of Artificial Sequence: Synthetic peptide"
PVPPPPP

SEQ ID NO: 83 - protein, 11 aa, Artificial Sequence
  source: /note="Description of Artificial Sequence: Synthetic peptide"
EDEDEDEDEDE

SEQ ID NO: 84 - protein, 14 aa, Artificial Sequence
  source: /note="Description of Artificial Sequence: Synthetic peptide"
DLPQETLEEETPGA

SEQ ID NO: 85 - protein, 12 aa, Artificial Sequence
  source: /note="Description of Artificial Sequence: Synthetic peptide"
VPSTPPTPSPST

SEQ ID NO: 86 - protein, 17 aa, Artificial Sequence
  source: /note="Description of Artificial Sequence: Synthetic peptide"
ELQLEESAAEAQEGELE

SEQ ID NO: 87 - protein, 18 aa, Artificial Sequence
  source: /note="Description of Artificial Sequence: Synthetic peptide"
ESPKAQASSVPTAQPQAE

SEQ ID NO: 88 - protein, 6 aa, Artificial Sequence
  source: /note="Description of Artificial Sequence: Synthetic peptide"
PAVPPP

SEQ ID NO: 89 - protein, 15 aa, Artificial Sequence
  source: /note="Description of Artificial Sequence: Synthetic peptide"
EPKSSDKTHTCPPCP

SEQ ID NO: 90 - protein, 13 aa, Artificial Sequence
  source: /note="Description of Artificial Sequence: Synthetic peptide"
VPSTPPTPSPSTG

SEQ ID NO: 91 - protein, 20 aa, Artificial Sequence
  source: /note="Description of Artificial Sequence: Synthetic peptide"
VPSTPPTPSPSTPPTPSPSG

SEQ ID NO: 92 - protein, 16 aa, Artificial Sequence
  source: /note="Description of Artificial Sequence: Synthetic peptide"
GRGGEEKKKEKEKEEG

SEQ ID NO: 93 - protein, 25 aa, Artificial Sequence
  source: /note="Description of Artificial Sequence: Synthetic peptide"
GRGGEEKKKEKEKEEQEERETKTPG

SEQ ID NO: 94 - protein, 10 aa, Artificial Sequence
  source: /note="Description of Artificial Sequence: Synthetic peptide"
ESPKAQASSG

SEQ ID NO: 95 - protein, 19 aa, Artificial Sequence
  source: /note="Description of Artificial Sequence: Synthetic peptide"
ESPKAQASSVPTAQPQAEG

SEQ ID NO: 96 - protein, 23 aa, Artificial Sequence
  source: /note="Description of Artificial Sequence: Synthetic peptide"
SVEEKKKEKEKEEQEERETKTPG

SEQ ID NO: 97 - protein, 24 aa, Artificial Sequence
  source: /note="Description of Artificial Sequence: Synthetic peptide"
PSVEEKKKEKEKEEQEERETKTPG

SEQ ID NO: 98 - protein, 24 aa, Artificial Sequence
  source: /note="Description of Artificial Sequence: Synthetic peptide"
GSVEEKKKEKEKEEQEERETKTPG

SEQ ID NO: 99 - protein, 232 aa, Artificial Sequence
  source: /note="Description of Artificial Sequence: Synthetic polypeptide"
EPRSSDKTHTCPPCPAPEAEGAPSVFLFPPKPKDTLMISRTPEVTCVVVDVSHEDPEVKFNWYVDGVEVHNAKTKPREEQYNSTYRVVSVLTVLHQDWLNGKEYKCKVSNKALPSSIEKTISKAKGQPREPQVYTLPPSRDELTKNQVSLTCLVKGFYPSDIAVEWESNGQPENNYKTTPPVLDSDGSFFLYSKLTVDKSRWQQGNVFSCSVMHEALHNHYTQKSLSLSPGK

SEQ ID NO: 100 - protein, 232 aa, Artificial Sequence
  source: /note="Description of Artificial Sequence: Synthetic polypeptide"
EPKSSDKTHTCPPCPAPEAEGAPSVFLFPPKPKDTLMISRTPEVTCVVVDVSHEDPEVKFNWYVDGVEVHNAKTKPREEQYNSTYRVVSVLTVLHQDWLNGKEYKCKVSNKALPSSIEKTISKAKGQPREPQVYTLPPSRDELTKNQVSLTCLVKGFYPSDIAVEWESNGQPENNYKTTPPVLDSDGSFFLYSKLTVDKSRWQQGNVFSCSVMHEALHNHYTQKSLSLSPGK

SEQ ID NO: 101 - protein, 231 aa, Artificial Sequence
  source: /note="Description of Artificial Sequence: Synthetic polypeptide"
EPKSSDKTHTCPPCPAPEAEGAPSVFLFPPKPKDTLMISRTPEVTCVVVDVSHEDPEVKFNWYVDGVEVHNAKTKPREEQYNSTYRVVSVLTVLHQDWLNGKEYKCKVSNKALPSSIEKTISKAKGQPREPQVYTLPPSRDELTKNQVSLTCLVKGFYPSDIAVEWESNGQPENNYKTTPPVLDSDGSFFLYSKLTVDKSRWQQGNVFSCSVMHEALHNHYTQKSLSLSPG

SEQ ID NO: 102 - protein, 232 aa, Artificial Sequence
  source: /note="Description of Artificial Sequence: Synthetic polypeptide"
EPKSCDKTHTCPPCPAPELLGGPSVFLFPPKPKDTLMISRTPEVTCVVVDVSHEDPEVKFNWYVDGVEVHNAKTKPREEQYQSTYRVVSVLTVLHQDWLNGKEYKCKVSNKALPAPIEKTISKAKGQPREPQVYTLPPSRDELTKNQVSLTCLVKGFYPSDIAVEWESNGQPENNYKTTPPVLDSDGSFFLYSKLTVDKSRWQQGNVFSCSVMHEALHNHYTQKSLSLSPGK

SEQ ID NO: 103 - protein, 232 aa, Artificial Sequence
  source: /note="Description of Artificial Sequence: Synthetic polypeptide"
EPRSSDKTHTCPPCPAPELLGGPSVFLFPPKPKDTLMISRTPEVTCVVVDVSHEDPEVKFNWYVDGVEVHNAKTKPREEQYNSTYRVVSVLTVLHQDWLNGKEYKCKVSNKALPAPIEKTISKAKGQPREPQVYTLPPSRDELTKNQVSLTCLVKGFYPSDIAVEWESNGQPENNYKTTPPVLDSDGSFFLYSKLTVDKSRWQQGNVFSCSVMHEALHNHYTQKSLSLSPGK

SEQ ID NO: 104 - protein, 227 aa, Artificial Sequence
  source: /note="Description of Artificial Sequence: Synthetic polypeptide"
DKTHTCPPCPAPELLGGPSVFLFPPKPKDTLMISRTPEVTCVVVDVSHEDPEVKFNWYVDGVEVHNAKTKPREEQYNSTYRVVSVLTVLHQDWLNGKEYKCKVSNKALPAPIEKTISKAKGQPREPQVYTLPPSRDELTKNQVSLTCLVKGFYPSDIAVEWESNGQPENNYKTTPPVLDSDGSFFLYSKLTVDKSRWQQGNVFSCSVMHEALHNHYTQKSLSLSPGK

SEQ ID NO: 105 - protein, 232 aa, Artificial Sequence
  source: /note="Description of Artificial Sequence: Synthetic polypeptide"
EPKSSDKTHTCPPCPAPELLGGPSVFLFPPKPKDTLMISRTPEVTCVVVDVSHEDPEVKFNWYVDGVEVHNAKTKPREEQYNSTYRVVSVLTVLHQDWLNGKEYKCKVSNKALPAPIEKTISKAKGQPREPQVYTLPPSRDELTKNQVSLTCLVKGFYPSDIAVEWESNGQPENNYKTTPPVLDSDGSFFLYSKLTVDKSRWQQGNVFSCSVMHEALHNHYTQKSLSLSPGK

SEQ ID NO: 106 - protein, 232 aa, Artificial Sequence
  source: /note="Description of Artificial Sequence: Synthetic polypeptide"
EPKSSDKTHTCPPCPAPEAEGAPSVFLFPPKPKDTLMISRTPEVTCVVVDVSHEDPEVKFNWYVDGVEVHNAKTKPREEQYNSTYRVVSVLTVLHQDWLNGKEYKCKVSNKALPAPIEKTISKAKGQPREPQVYTLPPSRDELTKNQVSLTCLVKGFYPSDIAVEWESNGQPENNYKTTPPVLDSDGSFFLYSKLTVDKSRWQQGNVFSCSVMHEALHNHYTQKSLSLSPGK

SEQ ID NO: 107 - protein, 232 aa, Artificial Sequence
  source: /note="Description of Artificial Sequence: Synthetic polypeptide"
EPKSSDKTHTSPPSPAPEAEGAPSVFLFPPKPKDTLMISRTPEVTCVVVDVSHEDPEVKFNWYVDGVEVHNAKTKPREEQYNSTYRVVSVLTVLHQDWLNGKEYKCKVSNKALPSSIEKTISKAKGQPREPQVYTLPPSRDELTKNQVSLTCLVKGFYPSDIAVEWESNGQPENNYKTTPPVLDSDGSFFLYSKLTVDKSRWQQGNVFSCSVMHEALHNHYTQKSLSLSPGK

SEQ ID NO: 108 - protein, 232 aa, Artificial Sequence
  source: /note="Description of Artificial Sequence: Synthetic polypeptide"
EPKSSDKTHTSPPSPAPEAEGAPSVFLFPPKPKDTLMISRTPEVTCVVVDVSHEDPEVKFNWYVDGVEVHNAKTKPREEQYNSTYRVVSVLTVLHQDWLNGKEYKCKVSNKALPSSIEKTISKAKGQPREPQVYTLPPSRDELTKNQVSLTCLVKGFYPSDIAVEWESNGQPENNYKTTPPVLDSDGSFFLGSKLTVDKSRWQQGNVFSCSVMHEALHNHYTQKSLSLSPGK

SEQ ID NO: 109 - protein, 232 aa, Artificial Sequence
  source: /note="Description of Artificial Sequence: Synthetic polypeptide"
EPKSSDKTHTSPPSPAPELLGGPSVFLFPPKPKDTLMISRTPEVTCVVVDVSHEDPEVKFNWYVDGVEVHNAKTKPREEQYNSTYRVVSVLTVLHQDWLNGKEYKCKVSNKALPAPIEKTISKAKGQPREPQVYTLPPSRDELTKNQVSLTCLVKGFYPSDIAVEWESNGQPENNYKTTPPVLDSDGSFFLGSKLTVDKSRWQQGNVFSCSVMHEALHNHYTQKSLSLSPGK

SEQ ID NO: 110 - protein, 229 aa, Artificial Sequence
  source: /note="Description of Artificial Sequence: Synthetic polypeptide"
ESKYGPPCPPCPAPEFLGGPSVFLFPPKPKDTLMISRTPEVTCVVVDVSQEDPEVKFNWYVDGVEVHNAKTKPREEQFNSTYRVVSVLTVLHQDWLNGKEYKCKVSNKGLPSSIEKTISKAKGQPREPQVYTLPPSQEEMTKNQVSLTCLVKGFYPSDIAVEWESNGQPENNYKTTPPVLDSDGSFFLYSRLTVDKSRWQEGNVFSCSVMHEALHNHYTQKSLSLSLGK

SEQ ID NO: 111 - protein, 232 aa, Artificial Sequence
  source: /note="Description of Artificial Sequence: Synthetic polypeptide"
EPKSSDKTHTCPPCPAPELLGGPSVFLFPPKPKDTLMISRTPEVTCVVVDVSHEDPEVKFNWYVDGVEVHNAKTKPREEQYNSTYRVVSVLTVLHQDWLNGKEYKCKVSNKALPAPIEKTISKAKGQPREPQVYTLPPSQEEMTKNQVSLTCLVKGFYPSDIAVEWESNGQPENNYKTTPPVLDSDGSFFLYSRLTVDKSRWQEGNVFSCSVMHEALHNHYTQKSLSLSLGK

SEQ ID NO: 112 - protein, 232 aa, Artificial Sequence
  source: /note="Description of Artificial Sequence: Synthetic polypeptide"
EPKSSDKTHTCPPCPAPELLGGPSVFLAPPKPKDTLMISRTPEVTCVVVDVSHEDPEVKFNWYVDGVEVHNAKTKPREEQYNSTYRVVSVLTVLHQDWLNGKEYKCKVSNKALPSSIEKTISKAKGQPREPQVYTLPPSRDELTKNQVSLTCLVKGFYPSDIAVEWESNGQPENNYKTTPPVLDSDGSFFLYSKLTVDKSRWQQGNVFSCSVMHEALHNHYTQKSLSLSPGK

SEQ ID NO: 113 - protein, 232 aa, Artificial Sequence
  source: /note="Description of Artificial Sequence: Synthetic polypeptide"
EPKSSDKTHTCPPCPAPELLGGPSVFLFPPKPKDTLMISRTPEVTCVVVDVSHEDPEVKFNWYVDGVEVHNAKTKPREEQYNSTYRVVSVLTVLHQDWLNGKEYKCKVSNKALPAPIEKTISKAKGQPREPQVYTLPPSRDELTKNQVSLTCLVKGFYPSDIAVEWESNGQPENNYKTTPPVLDSDGSFFLYSKLTVDKSRWQQGNVFSCSVMHEALHNAYTQKSLSLSPGK

SEQ ID NO: 114 - protein, 232 aa, Artificial Sequence
  source: /note="Description of Artificial Sequence: Synthetic polypeptide"
EPKSSDKTHTCPPCPAPEAEGAPSVFLFPPKPKDTLMISRTPEVTCVVVDVSHEDPEVKFNWYVDGVEVHNAKTKPREEQYQSTYRVVSVLTVLHQDWLNGKEYKCKVSNKALPSSIEKTISKAKGQPREPQVYTLPPSRDELTKNQVSLTCLVKGFYPSDIAVEWESNGQPENNYKTTPPVLDSDGSFFLYSKLTVDKSRWQQGNVFSCSVMHEALHNHYTQKSLSLSPGK

SEQ ID NO: 115 - protein, 232 aa, Artificial Sequence
  source: /note="Description of Artificial Sequence: Synthetic polypeptide"
EPKSSDKTHTSPPSPAPEAEGAPSVFLFPPKPKDTLMISRTPEVTCVVVDVSHEDPEVKFNWYVDGVEVHNAKTKPREEQYNSTYRVVSVLTVLHQDWLNGKEYKCKVSNKALPSSIEKTISKAKGQPREPQVYTLPPSRDELTKNQVSLTCLVKGFYPSDIAVEWESNGQPENNYKTTPPVLDSDGSFALGSKLTVDKSRWQQGNVFSCSVMHEALHNHYTQKSLSLSPGK

SEQ ID NO: 116 - protein, 232 aa, Artificial Sequence
  source: /note="Description of Artificial Sequence: Synthetic polypeptide"
EPKSSDKTHTSPPSPAPELLGGPSVFLFPPKPKDTLMISRTPEVTCVVVDVSHEDPEVKFNWYVDGVEVHNAKTKPREEQYNSTYRVVSVLTVLHQDWLNGKEYKCKVSNKALPAPIEKTISKAKGQPREPQVYTLPPSRDELTKNQVSLTCLVKGFYPSDIAVEWESNGQPENNYKTTPPVLDSDGSFALGSKLTVDKSRWQQGNVFSCSVMHEALHNHYTQKSLSLSPGK

SEQ ID NO: 117 - protein, 232 aa, Artificial Sequence
  source: /note="Description of Artificial Sequence: Synthetic polypeptide"
EPKSSDKTHTCPPCPAPEAGGGPSVFLFPPKPKDTLMISRTPEVTCVVVDVSHEDPEVKFNWYVDGVEVHNAKTKPREEQYNSTYRVVSVLTVLHQDWLNGKEYKCKVSNKALPASIEKTISKAKGQPREPQVYTLPPSRDELTKNQVSLTCLVKGFYPSDIAVEWESNGQPENNYKTTPPVLDSDGSFFLYSKLTVDKSRWQQGNVFSCSVMHEALHNHYTQKSLSLSPGK

SEQ ID NO: 118 - protein, 233 aa, Mus sp.
EPRGPTIKPCPPCKCPAPNLLGGPSVFIFPPKIKDVLMISLSPIVTCVVVDVSEDDPDVQISWFVNNVEVHTAQTQTHREDYNSTLRVVSALPIQHQDWMSGKEFKCKVNNKDLPAPIERTISKPKGSVRAPQVYVLPPPEEEMTKKQVTLTCMVTDFMPEDIYVEWTNNGKTELNYKNTEPVLDSDGSYFMYSKLRVEKKNWVERNSYSCSVVHEGLHNHHTTKSFSRTPGK

SEQ ID NO: 119 - protein, 238 aa, Mus sp.
EPRVPITQNPCPPLKECPPCAAPDLLGGPSVFIFPPKIKDVLMISLSPMVTCVVVDVSEDDPDVQISWFVNNVEVHTAQTQTHREDYNSTLRVVSALPIQHQDWMSGKEFKCKVNNRALPSPIEKTISKPRGPVRAPQVYVLPPPAEEMTKKEFSLTCMITGFLPAEIAVDWTSNGRTEQNYKNTATVLDSDGSYFMYSKLRVQKSTWERGSLFACSVVHEGLHNHLTTKTISRSLGK

SEQ ID NO: 120 - protein, 233 aa, Artificial Sequence
  source: /note="Description of Artificial Sequence: Synthetic polypeptide"
EPRSPTIKPCPPCKCPAPNLEGGPSVFIFPPKIKDVLMISLSPIVTCVVVDVSEDDPDVQISWFVNNVEVHTAQTQTHREDYNSTLRVVSALPIQHQDWMSGKAFACAVNNKDLPAPIERTISKPKGSVRAPQVYVLPPPEEEMTKKQVTLTCMVTDFMPEDIYVEWTNNGKTELNYKNTEPVLDSDGSYFMYSKLRVEKKNWVERNSYSCSVVHEGLHNHHTTKSFSRTPGK

SEQ ID NO: 121 - protein, 238 aa, Artificial Sequence
  source: /note="Description of Artificial Sequence: Synthetic polypeptide"
EPRSPITQNPCPPLKECPPCAAPDLEGGPSVFIFPPKIKDVLMISLSPMVTCVVVDVSEDDPDVQISWFVNNVEVHTAQTQTHREDYNSTLRVVSALPIQHQDWMSGKAFACAVNNRALPSPIEKTISKPRGPVRAPQVYVLPPPAEEMTKKEFSLTCMITGFLPAEIAVDWTSNGRTEQNYKNTATVLDSDGSYFMYSKLRVQKSTWERGSLFACSVVHEGLHNHLTTKTISRSLGK

SEQ ID NO: 122 - protein, 329 aa, Artificial Sequence
  source: /note="Description of Artificial Sequence: Synthetic polypeptide"
GVSDVPRDLEVVAATPTSLLISWRPPIHAYGYYRITYGETGGNSPVQEFTVPIVEGTATISGLKPGVDYTITVYAVEYTFKHSGYYHRPISINYRTEIEPKSSGSTHTCPPCPAPELLGGSSVFLFPPKPKDTLMISRTPEVTCVVVDVSHEDPEVKFNWYVDGVEVHNAKTKPREEQYNSTYRVVSVLTVLHQDWLNGKEYKCKVSNKALPAPIEKTISKAKGQPREPQVYTLPPSRDELTKNQVSLTCLVKGFYPSDIAVEWESNGQPENNYKTTPPVLDSDGSFFLYSKLTVDKSRWQQGNVFSCSVMHEALHNHYTQKSLSLSPG

SEQ ID NO: 123 - protein, 336 aa, Artificial Sequence
  source: /note="Description of Artificial Sequence: Synthetic polypeptide"
EPKSSGSTHTCPPCPAPELLGGSSVFLFPPKPKDTLMISRTPEVTCVVVDVSHEDPEVKFNWYVDGVEVHNAKTKPREEQYNSTYRVVSVLTVLHQDWLNGKEYKCKVSNKALPAPIEKTISKAKGQPREPQVYTLPPSRDELTKNQVSLTCLVKGFYPSDIAVEWESNGQPENNYKTTPPVLDSDGSFFLYSKLTVDKSRWQQGNVFSCSVMHEALHNHYTQKSLSLSPGAGGGGSGGVSDVPRDLEVVAATPTSLLISWRPPIHAYGYYRITYGETGGNSPVQEFTVPIVEGTATISGLKPGVDYTITVYAVEYTFKHSGYYHRPISINYRTEI

SEQ ID NO: 124 - protein, 329 aa, Artificial Sequence
  source: /note="Description of Artificial Sequence: Synthetic polypeptide"
GVSDVPRDLEVVAATPTSLLISWSPPANGYGYYRITYGETGGNSPVQEFTVPVGRGTATISGLKPGVDYTITVYAVEYTYKGSGYYHRPISINYRTEIEPKSSGSTHTCPPCPAPELLGGSSVFLFPPKPKDTLMISRTPEVTCVVVDVSHEDPEVKFNWYVDGVEVHNAKTKPREEQYNSTYRVVSVLTVLHQDWLNGKEYKCKVSNKALPAPIEKTISKAKGQPREPQVYTLPPSRDELTKNQVSLTCLVKGFYPSDIAVEWESNGQPENNYKTTPPVLDSDGSFFLYSKLTVDKSRWQQGNVFSCSVMHEALHNHYTQKSLSLSPG

SEQ ID NO: 125 - protein, 336 aa, Artificial Sequence
  source: /note="Description of Artificial Sequence: Synthetic polypeptide"
EPKSSGSTHTCPPCPAPELLGGSSVFLFPPKPKDTLMISRTPEVTCVVVDVSHEDPEVKFNWYVDGVEVHNAKTKPREEQYNSTYRVVSVLTVLHQDWLNGKEYKCKVSNKALPAPIEKTISKAKGQPREPQVYTLPPSRDELTKNQVSLTCLVKGFYPSDIAVEWESNGQPENNYKTTPPVLDSDGSFFLYSKLTVDKSRWQQGNVFSCSVMHEALHNHYTQKSLSLSPGAGGGGSGGVSDVPRDLEVVAATPTSLLISWSPPANGYGYYRITYGETGGNSPVQEFTVPVGRGTATISGLKPGVDYTITVYAVEYTYKGSGYYHRPISINYRTEI

SEQ ID NO: 126 - protein, 329 aa, Artificial Sequence
  source: /note="Description of Artificial Sequence: Synthetic polypeptide"
GVSDVPRDLEVVAATPTSLLISWGHYPLHVRYYRITYGETGGNSPVQEFTVPPRSHTATISGLKPGVDYTITVYAVTYYAQENYKEIPISINYRTEIEPKSSGSTHTCPPCPAPELLGGSSVFLFPPKPKDTLMISRTPEVTCVVVDVSHEDPEVKFNWYVDGVEVHNAKTKPREEQYNSTYRVVSVLTVLHQDWLNGKEYKCKVSNKALPAPIEKTISKAKGQPREPQVYTLPPSRDELTKNQVSLTCLVKGFYPSDIAVEWESNGQPENNYKTTPPVLDSDGSFFLYSKLTVDKSRWQQGNVFSCSVMHEALHNHYTQKSLSLSPGK

SEQ ID NO: 127 - protein, 336 aa, Artificial Sequence
  source: /note="Description of Artificial Sequence: Synthetic polypeptide"
EPKSSGSTHTCPPCPAPELLGGSSVFLFPPKPKDTLMISRTPEVTCVVVDVSHEDPEVKFNWYVDGVEVHNAKTKPREEQYNSTYRVVSVLTVLHQDWLNGKEYKCKVSNKALPAPIEKTISKAKGQPREPQVYTLPPSRDELTKNQVSLTCLVKGFYPSDIAVEWESNGQPENNYKTTPPVLDSDGSFFLYSKLTVDKSRWQQGNVFSCSVMHEALHNHYTQKSLSLSPGAGGGGSGGVSDVPRDLEVVAATPTSLLISWGHYPLHVRYYRITYGETGGNSPVQEFTVPPRSHTATISGLKPGVDYTITVYAVTYYAQENYKEIPISINYRTEAS

SEQ ID NO: 128 - protein, 330 aa, Artificial Sequence
  source: /note="Description of Artificial Sequence: Synthetic polypeptide"
GSVSDVPRDLEVVAATPTSLLISWRHPHFPTRYYRITYGETGGNSPVQEFTVPLQPPTATISGLKPGVDYTITVYAVTDGRNGRLLSIPISINYRTEIEPKSSDKTHTCPPCPAPELLGGSSVFLFPPKPKDTLMISRTPEVTCVVVDVSHEDPEVKFNWYVDGVEVHNAKTKPREEQYNSTYRVVSVLTVLHQDWLNGKEYKCKVSNKALPAPIEKTISKAKGQPREPQVYTLPPSRDELTKNQVSLTCLVKGFYPSDIAVEWESNGQPENNYKTTPPVLDSDGSFFLYSKLTVDKSRWQQGNVFSCSVMHEALHNHYTQKSLSLSPGK

SEQ ID NO: 129 - protein, 330 aa, Artificial Sequence
  source: /note="Description of Artificial Sequence: Synthetic polypeptide"
GSVSDVPRDLEVVAATPTSLLISWRHPHFPTRYYRITYGETGGNSPVQEFTVPLQPPTATISGLKPGVDYTITVYAVTDGRNGRLLSIPISINYRTEIEPKSSDKTHTCPPCPAPELLGGPSVFLFPPKPKDTLMISRTPEVTCVVVDVSHEDPEVKFNWYVDGVEVHNAKTKPREEQYNSTYRVVSVLTVLHQDWLNGKEYKCKVSNKALPAPIEKTISKAKGQPREPQVYTLPPSRDELTKNQVSLTCLVKGFYPSDIAVEWESNGQPENNYKTTPPVLDSDGSFFLYSKLTVDKSRWQQGNVFSCSVMHEALHNHYTQKSLSLSPGK

SEQ ID NO: 130 - protein, 5 aa, Artificial Sequence
  source: /note="Description of Artificial Sequence: Synthetic peptide"
GGGGS

SEQ ID NO: 131 - protein, 22 aa, Artificial Sequence
  source: /note="Description of Artificial Sequence: Synthetic peptide"
  VARIANT (1)..(1): /replace=" "
  VARIANT (2)..(2): /replace=" "
  misc_feature (1)..(2): /note="Residues given in the sequence have no preference with respect to those in the annotations for said positions"
  misc_feature (3)..(22): /note="This region may encompass 2 to 10 'Glu Asp' repeating units"
EIEDEDEDEDEDEDEDEDEDED

SEQ ID NO: 132 - protein, 7 aa, Artificial Sequence
  source: /note="Description of Artificial Sequence: Synthetic peptide"
ELQLEES

SEQ ID NO: 133 - protein, 21 aa, Artificial Sequence
  source: /note="Description of Artificial Sequence: Synthetic peptide"
QKSLSLSPQPDEPGVSDVPRD

SEQ ID NO: 134 - protein, 23 aa, Artificial Sequence
  source: /note="Description of Artificial Sequence: Synthetic peptide"
QKSLSLSPAGGGGSGGVSDVPRD

SEQ ID NO: 135 - protein, 23 aa, Artificial Sequence
  source: /note="Description of Artificial Sequence: Synthetic peptide"
QKSLSLSPPVPPPPPGVSDVPRD

SEQ ID NO: 136 - protein, 27 aa, Artificial Sequence
  source: /note="Description of Artificial Sequence: Synthetic peptide"
QKSLSLSPEDEDEDEDEDEGVSDVPRD

SEQ ID NO: 137 - protein, 30 aa, Artificial Sequence
  source: /note="Description of Artificial Sequence: Synthetic polypeptide"
QKSLSLSPDLPQETLEEETPGAGVSDVPRD

SEQ ID NO: 138 - protein, 28 aa, Artificial Sequence
  source: /note="Description of Artificial Sequence: Synthetic peptide"
QKSLSLSPVPSTPPTPSPSTGVSDVPRD

SEQ ID NO: 139 - protein, 33 aa, Artificial Sequence
  source: /note="Description of Artificial Sequence: Synthetic polypeptide"
QKSLSLSPELQLEESAAEAQEGELEGVSDVPRD

SEQ ID NO: 140 - protein, 34 aa, Artificial Sequence
  source: /note="Description of Artificial Sequence: Synthetic polypeptide"
QKSLSLSPESPKAQASSVPTAQPQAEGVSDVPRD

SEQ ID NO: 141 - protein, 22 aa, Artificial Sequence
  source: /note="Description of Artificial Sequence: Synthetic peptide"
QKSLSLSPPAVPPPGVSDVPRD

SEQ ID NO: 142 - protein, 23 aa, Artificial Sequence
  source: /note="Description of Artificial Sequence: Synthetic peptide"
QKSLSLSPELQLEESGVSDVPRD

SEQ ID NO: 143 - protein, 33 aa, Artificial Sequence; identical to SEQ ID NO: 139
  source: /note="Description of Artificial Sequence: Synthetic polypeptide"

SEQ ID NO: 144 - protein, 29 aa, Artificial Sequence
  source: /note="Description of Artificial Sequence: Synthetic peptide"
QKSLSLSPVPSTPPTPSPSTGGVSDVPRD

SEQ ID NO: 145 - protein, 36 aa, Artificial Sequence
  source: /note="Description of Artificial Sequence: Synthetic polypeptide"
QKSLSLSPVPSTPPTPSPSTPPTPSPSGGVSDVPRD

SEQ ID NO: 146 - protein, 32 aa, Artificial Sequence
  source: /note="Description of Artificial Sequence: Synthetic polypeptide"
QKSLSLSPGRGGEEKKKEKEKEEGGVSDVPRD

SEQ ID NO: 147 - protein, 41 aa, Artificial Sequence
  source: /note="Description of Artificial Sequence: Synthetic polypeptide"
QKSLSLSPGRGGEEKKKEKEKEEQEERETKTPGGVSDVPRD

SEQ ID NO: 148 - protein, 26 aa, Artificial Sequence
  source: /note="Description of Artificial Sequence: Synthetic peptide"
QKSLSLSPESPKAQASSGGVSDVPRD

SEQ ID NO: 149 - protein, 35 aa, Artificial Sequence
  source: /note="Description of Artificial Sequence: Synthetic polypeptide"
QKSLSLSPESPKAQASSVPTAQPQAEGGVSDVPRD

SEQ ID NO: 150 - protein, 39 aa, Artificial Sequence
  source: /note="Description of Artificial Sequence: Synthetic polypeptide"
QKSLSLSPSVEEKKKEKEKEEQEERETKTPGGVSDVPRD

SEQ ID NO: 151 - protein, 40 aa, Artificial Sequence
  source: /note="Description of Artificial Sequence: Synthetic polypeptide"
QKSLSLSPPSVEEKKKEKEKEEQEERETKTPGGVSDVPRD

SEQ ID NO: 152 - protein, 40 aa, Artificial Sequence
  source: /note="Description of Artificial Sequence: Synthetic polypeptide"
QKSLSLSPGSVEEKKKEKEKEEQEERETKTPGGVSDVPRD

SEQ ID NO: 153 - protein, 6 aa, Artificial Sequence
  source: /note="Description of Artificial Sequence: Synthetic 6xHis tag"
HHHHHH

SEQ ID NO: 154 - protein, 232 aa, Homo sapiens
EPKSCDKTHTCPPCPAPELLGGPSVFLFPPKPKDTLMISRTPEVTCVVVDVSHEDPEVKFNWYVDGVEVHNAKTKPREEQYNSTYRVVSVLTVLHQDWLNGKEYKCKVSNKALPAPIEKTISKAKGQPREPQVYTLPPSRDELTKNQVSLTCLVKGFYPSDIAVEWESNGQPENNYKTTPPVLDSDGSFFLYSKLTVDKSRWQQGNVFSCSVMHEALHNHYTQKSLSLSPGK